European Patent Specification EP 3 649 152 B1, published October 8, 2025. Title: ROR1 Antibodies. Applicant: UCL Business PLC. The sequence listing filed with the application follows.

SEQUENCE LISTING (313 sequences)

SEQ ID NO: 1 - protein, 26 aa, Rattus norvegicus
DVVMTQTPVSLPVSLGGQVSISCRSS

SEQ ID NO: 2 - protein, 11 aa, Rattus norvegicus
QSLEHSNGDTF

SEQ ID NO: 3 - protein, 17 aa, Rattus norvegicus
LHWYLQKPGQSPRLLIY

SEQ ID NO: 4 - protein, 3 aa, Rattus norvegicus
RVS

SEQ ID NO: 5 - protein, 36 aa, Rattus norvegicus
NRFSGVPDRFSGSGSGTDFTLKISRIEPEDLGDYYC

SEQ ID NO: 6 - protein, 9 aa, Rattus norvegicus
LQSTHFPNT

SEQ ID NO: 7 - protein, 10 aa, Rattus norvegicus
FGAGTKLELK

SEQ ID NO: 8 - protein, 26 aa, Rattus norvegicus
DIQLTQSPSTLSASLGERVTISCRAS

SEQ ID NO: 9 - protein, 6 aa, Rattus norvegicus
QSISNS

SEQ ID NO: 10 - protein, 17 aa, Rattus norvegicus
LNWYQQKPDGTVKRLIY

SEQ ID NO: 11 - protein, 3 aa, Rattus norvegicus
STS

SEQ ID NO: 12 - protein, 36 aa, Rattus norvegicus
TLESGVPSRFSGSGSGTDFSLSISSLESEDFAMYYC

SEQ ID NO: 13 - protein, 10 aa, Rattus norvegicus
LQFATYPQVT

SEQ ID NO: 14 - protein, 10 aa, Rattus norvegicus
FGSGTKLEIK

SEQ ID NO: 15 - protein, 25 aa, Rattus norvegicus
DIVLTQSPALAVSVGQRATISCRAS

SEQ ID NO: 16 - protein, 10 aa, Rattus norvegicus
QSVSISRYNF

SEQ ID NO: 17 - protein, 17 aa, Rattus norvegicus
MHWYQQKPGQQPKLLIY

SEQ ID NO: 18 - protein, 3 aa, Rattus norvegicus
RAS

SEQ ID NO: 19 - protein, 36 aa, Rattus norvegicus
NLASGIPARFSGSGSGTDFTLTINPVQADDIATYYC

SEQ ID NO: 20 - protein, 9 aa, Rattus norvegicus
QQNRESPRT

SEQ ID NO: 21 - protein, 10 aa, Rattus norvegicus
FGGGTKLELK

SEQ ID NO: 22 - protein, 10 aa, Rattus norvegicus
QSVSISRYDF

SEQ ID NO: 23 - protein, 26 aa, Rattus norvegicus
DIQMTQSPSFLSASVGDRVTINCKAS

SEQ ID NO: 24 - protein, 6 aa, Rattus norvegicus
QNIDRY

SEQ ID NO: 25 - protein, 17 aa, Rattus norvegicus
LNWYQQKLGEAPKRLLY

SEQ ID NO: 26 - protein, 3 aa, Rattus norvegicus
NTN

SEQ ID NO: 27 - protein, 36 aa, Rattus norvegicus
KLQTGIPSRFSGSGSATDFTLTISSLQPEDFATYFC

SEQ ID NO: 28 - protein, 9 aa, Rattus norvegicus
LQYNSLPLT

SEQ ID NO: 29 - protein, 26 aa, Rattus norvegicus
DIQMTQSPSSMSASLGDRVTFTCQAS

SEQ ID NO: 30 - protein, 6 aa, Rattus norvegicus
QDIGNN

SEQ ID NO: 31 - protein, 17 aa, Rattus norvegicus
LIWFQQKPGKSPRPLMY

SEQ ID NO: 32 - protein, 3 aa, Rattus norvegicus
FAT

SEQ ID NO: 33 - protein, 36 aa, Rattus norvegicus
SLANGVPSRFSGSRSGSDYSLTISSLESEDLADYHC

SEQ ID NO: 34 - protein, 9 aa, Rattus norvegicus
LQYREYPLT

SEQ ID NO: 35 - protein, 10 aa, Rattus norvegicus
FGSGTKLDLK

SEQ ID NO: 36 - protein, 26 aa, Rattus norvegicus
DIRMTQSPASLSASLGETVTIECLTS

SEQ ID NO: 37 - protein, 6 aa, Rattus norvegicus
EDIYSD

SEQ ID NO: 38 - protein, 17 aa, Rattus norvegicus
LAWFQQKPGKSPQLLIY

SEQ ID NO: 39 - protein, 3 aa, Rattus norvegicus
DAN

SEQ ID NO: 40 - protein, 36 aa, Rattus norvegicus
SLQNGVPSRFGGCGSGTQYSLQISSLQSEDVATYFC

SEQ ID NO: 41 - protein, 9 aa, Rattus norvegicus
QQYKNYPPT

SEQ ID NO: 42 - protein, 10 aa, Rattus norvegicus
FGGGTKLVLK

SEQ ID NO: 43 - protein, 26 aa, Rattus norvegicus
DIQLTQSPSSMSASLGDRVSLTCQSS

SEQ ID NO: 44 - protein, 6 aa, Rattus norvegicus
QGIGKY

SEQ ID NO: 45 - protein, 17 aa, Rattus norvegicus
LSWYQHKPGKPPKAMIY

SEQ ID NO: 46 - protein, 3 aa, Rattus norvegicus
YAT

SEQ ID NO: 47 - protein, 36 aa, Rattus norvegicus
KLADGVPSRFSGSRSGSDFSLTISSLESEDIAIYYC

SEQ ID NO: 48 - protein, 9 aa, Rattus norvegicus
LQFDDYPWT

SEQ ID NO: 49 - protein, 25 aa, Rattus norvegicus
DIVLTQSPALAVSLEQRVTIACKTS

SEQ ID NO: 50 - protein, 10 aa, Rattus norvegicus
QNVDNHGISY

SEQ ID NO: 51 - protein, 17 aa, Rattus norvegicus
MHWYQQKSGQEPKLLIY

SEQ ID NO: 52 - protein, 3 aa, Rattus norvegicus
EGS

SEQ ID NO: 53 - protein, 36 aa, Rattus norvegicus
NLAVGIPARFSGSGSGTDFTLTIDPVEADDIETYYC

SEQ ID NO: 54 - protein, 9 aa, Rattus norvegicus
QQSKDDPRT

SEQ ID NO: 55 - protein, 25 aa, Rattus norvegicus
QFTLTQPKSVSGSLRSTITIPCERS

SEQ ID NO: 56 - protein, 8 aa, Rattus norvegicus
SGDIGDSY

SEQ ID NO: 57 - protein, 17 aa, Rattus norvegicus
VSWYQQHLGRPPINVIY

SEQ ID NO: 58 - protein, 3 aa, Rattus norvegicus
ADD

SEQ ID NO: 59 - protein, 38 aa, Rattus norvegicus
QRPSEVSDRFSGSIDSSSNSASLTITNLQMDDEADYFC

SEQ ID NO: 60 - protein, 12 aa, Rattus norvegicus
QSYDRNVDFNTV

SEQ ID NO: 61 - protein, 10 aa, Rattus norvegicus
FGGGTKVTVL

SEQ ID NO: 62 - protein, 26 aa, Rattus norvegicus
DIQLTQSPSSLSASLGDRVSLTCQSS

SEQ ID NO: 63 - protein, 17 aa, Rattus norvegicus
LSWFQHKPGKPPKPVIN

SEQ ID NO: 64 - protein, 36 aa, Rattus norvegicus
NLADGVPSRFSGRRSGSDFSLTISSLESEDTAIYYC

SEQ ID NO: 65 - protein, 9 aa, Rattus norvegicus
LQFDDFRWT

SEQ ID NO: 66 - protein, 10 aa, Rattus norvegicus
VGGGTKLELK

SEQ ID NO: 67 - protein, 8 aa, Rattus norvegicus
SGDIGDNY

SEQ ID NO: 68 - protein, 11 aa, Rattus norvegicus
QSFDSNFDIPV

SEQ ID NO: 69 - protein, 10 aa, Rattus norvegicus
FGGGTKLTVL

SEQ ID NO: 70 - protein, 26 aa, Rattus norvegicus
DIKMTQSPSFLSASVGDRVTINCKAS

SEQ ID NO: 71 - protein, 6 aa, Rattus norvegicus
QNITRF

SEQ ID NO: 72 - protein, 17 aa, Rattus norvegicus
LNWYQQELGEAPTLLIY

SEQ ID NO: 73 - protein, 36 aa, Rattus norvegicus
NLQTGIPSRFSGSGSGTDFTLTISSLQPEDVATYFC

SEQ ID NO: 74 - protein, 9 aa, Rattus norvegicus
LQHGSRPRT

SEQ ID NO: 75 - protein, 112 aa, Rattus norvegicus
DVVMTQTPVSLPVSLGGQVSISCRSSQSLEHSNGDTFLHWYLQKPGQSPRLLIYRVSNRFSGVPDRFSGSGSGTDFTLKISRIEPEDLGDYYCLQSTHFPNTFGAGTKLELK

SEQ ID NO: 76 - protein, 108 aa, Rattus norvegicus
DIQLTQSPSTLSASLGERVTISCRASQSISNSLNWYQQKPDGTVKRLIYSTSTLESGVPSRFSGSGSGTDFSLSISSLESEDFAMYYCLQFATYPQVTFGSGTKLEIK

SEQ ID NO: 77 - protein, 110 aa, Rattus norvegicus
DIVLTQSPALAVSVGQRATISCRASQSVSISRYNFMHWYQQKPGQQPKLLIYRASNLASGIPARFSGSGSGTDFTLTINPVQADDIATYYCQQNRESPRTFGGGTKLELK

SEQ ID NO: 78 - protein, 110 aa, Rattus norvegicus
DIVLTQSPALAVSVGQRATISCRASQSVSISRYDFMHWYQQKPGQQPKLLIYRASNLASGIPARFSGSGSGTDFTLTINPVQADDIATYYCQQNRESPRTFGGGTKLELK

SEQ ID NO: 79 - protein, 107 aa, Rattus norvegicus
DIQMTQSPSFLSASVGDRVTINCKASQNIDRYLNWYQQKLGEAPKRLLYNTNKLQTGIPSRFSGSGSATDFTLTISSLQPEDFATYFCLQYNSLPLTFGSGTKLEIK

SEQ ID NO: 80 - protein, 107 aa, Rattus norvegicus
DIQMTQSPSSMSASLGDRVTFTCQASQDIGNNLIWFQQKPGKSPRPLMYFATSLANGVPSRFSGSRSGSDYSLTISSLESEDLADYHCLQYREYPLTFGSGTKLDLK

SEQ ID NO: 81 - protein, 107 aa, Rattus norvegicus
DIRMTQSPASLSASLGETVTIECLTSEDIYSDLAWFQQKPGKSPQLLIYDANSLQNGVPSRFGGCGSGTQYSLQISSLQSEDVATYFCQQYKNYPPTFGGGTKLVLK

SEQ ID NO: 82 - protein, 107 aa, Rattus norvegicus
DIQLTQSPSSMSASLGDRVSLTCQSSQGIGKYLSWYQHKPGKPPKAMIYYATKLADGVPSRFSGSRSGSDFSLTISSLESEDIAIYYCLQFDDYPWTFGGGTKLELK

SEQ ID NO: 83 - protein, 110 aa, Rattus norvegicus
DIVLTQSPALAVSLEQRVTIACKTSQNVDNHGISYMHWYQQKSGQEPKLLIYEGSNLAVGIPARFSGSGSGTDFTLTIDPVEADDIETYYCQQSKDDPRTFGGGTKLELK

SEQ ID NO: 84 - protein, 113 aa, Rattus norvegicus
QFTLTQPKSVSGSLRSTITIPCERSSGDIGDSYVSWYQQHLGRPPINVIYADDQRPSEVSDRFSGSIDSSSNSASLTITNLQMDDEADYFCQSYDRNVDFNTVFGGGTKVTVL

SEQ ID NO: 85 - protein, 107 aa, Rattus norvegicus
DIQLTQSPSSLSASLGDRVSLTCQSSQGIGKYLSWFQHKPGKPPKPVINYATNLADGVPSRFSGRRSGSDFSLTISSLESEDTAIYYCLQFDDFRWTVGGGTKLELK

SEQ ID NO: 86 - protein, 112 aa, Rattus norvegicus
QFTLTQPKSVSGSLRSTITIPCERSSGDIGDNYVSWYQQHLGRPPINVIYADDQRPSEVSDRFSGSIDSSSNSASLTITNLQMDDEADYFCQSFDSNFDIPVFGGGTKLTVL

SEQ ID NO: 87 - protein, 107 aa, Rattus norvegicus
DIKMTQSPSFLSASVGDRVTINCKASQNITRFLNWYQQELGEAPTLLIYNTNNLQTGIPSRFSGSGSGTDFTLTISSLQPEDVATYFCLQHGSRPRTFGGGTKLELK

SEQ ID NO: 88 - protein, 25 aa, Rattus norvegicus
EVQLQESGPGLVKPAQSLSLTCSVT

SEQ ID NO: 89 - protein, 9 aa, Rattus norvegicus
GYSITNMYR

SEQ ID NO: 90 - protein, 17 aa, Rattus norvegicus
WNWIRKFPGNKLEWMGY

SEQ ID NO: 91 - protein, 7 aa, Rattus norvegicus
INTAGST

SEQ ID NO: 92 - protein, 38 aa, Rattus norvegicus
DYSPSLRGRVSITGDTSKNQFFLHLTSVTTEDTATYYC

SEQ ID NO: 93 - protein, 10 aa, Rattus norvegicus
AGFITNPFDF

SEQ ID NO: 94 - protein, 11 aa, Rattus norvegicus
WGQGVMVTVSS

SEQ ID NO: 95 - protein, 25 aa, Rattus norvegicus
EVQVVESGGGLVQPGRSLKLSCVPS

SEQ ID NO: 96 - protein, 8 aa, Rattus norvegicus
GFTFNNYW

SEQ ID NO: 97 - protein, 17 aa, Rattus norvegicus
MTWIRQAPGKAPEWVAS

SEQ ID NO: 98 - protein, 8 aa, Rattus norvegicus
ISNTGGST

SEQ ID NO: 99 - protein, 38 aa, Rattus norvegicus
FYPDSVRGRFSISRDNTKGTLYLHMTSLRSEDTATYYC

SEQ ID NO: 100 - protein, 6 aa, Rattus norvegicus
IRNMDA

SEQ ID NO: 101 - protein, 11 aa, Rattus norvegicus
WGQGTSVTVSS

SEQ ID NO: 102 - protein, 24 aa, Rattus norvegicus
GKLVESGGGLLKPGGSLKLSCVAS

SEQ ID NO: 103 - protein, 8 aa, Rattus norvegicus
GFTFDKYW

SEQ ID NO: 104 - protein, 17 aa, Rattus norvegicus
MHWVRQAPGKGLEWIAE

SEQ ID NO: 105 - protein, 8 aa, Rattus norvegicus
IEYDGTET

SEQ ID NO: 106 - protein, 38 aa, Rattus norvegicus
NYAPSIKDRFTISRDNAKNTLYLQMSNVRSEDAATYFC

SEQ ID NO: 107 - protein, 16 aa, Rattus norvegicus
TTEEMYTTDYYYGFAY

SEQ ID NO: 108 - protein, 11 aa, Rattus norvegicus
WGQGTLVTVSS

SEQ ID NO: 109 - protein, 25 aa, Rattus norvegicus
DVKLVESGGGLLKPGGSLKLSCVAS

SEQ ID NO: 110 - protein, 8 aa, Rattus norvegicus
GFSFSKYW

SEQ ID NO: 111 - protein, 17 aa, Rattus norvegicus
MHWVRQAPGQGLEWIAE

SEQ ID NO: 112 - protein, 38 aa, Rattus norvegicus
NYAPSIKDRFTISRDNAKNTLYLQMSNVRFEDAATYFC

SEQ ID NO: 113 - protein, 16 aa, Rattus norvegicus
TTEEMHTTDYYYGFAY

SEQ ID NO: 114 - protein, 25 aa, Rattus norvegicus
EVQLVESGGGLVQPGRSLKLSCAAS

SEQ ID NO: 115 - protein, 8 aa, Rattus norvegicus
GFIFSEHN

SEQ ID NO: 116 - protein, 17 aa, Rattus norvegicus
MAWVRQAPKKGLEWVAT

SEQ ID NO: 117 - protein, 8 aa, Rattus norvegicus
ISDDGRNT

SEQ ID NO: 118 - protein, 38 aa, Rattus norvegicus
YYRDSMRGRFTISRENARSTLYLQLDSLRSEDTATYYC

SEQ ID NO: 119 - protein, 10 aa, Rattus norvegicus
ASHRYNLFDS

SEQ ID NO: 120 - protein, 25 aa, Rattus norvegicus
QVQLQQSGTELVKPASSVRISCKAS

SEQ ID NO: 121 - protein, 8 aa, Rattus norvegicus
GYTLTTNY

SEQ ID NO: 122 - protein, 17 aa, Rattus norvegicus
MHWIRQQPGNGLEWIGW

SEQ ID NO: 123 - protein, 8 aa, Rattus norvegicus
IYPGNGNT

SEQ ID NO: 124 - protein, 38 aa, Rattus norvegicus
KFNHKFDGRTTLTADKSSSIVYMQLSSLTSEDSAVYFC

SEQ ID NO: 125 - protein, 7 aa, Rattus norvegicus
ARSDFDY

SEQ ID NO: 126 - protein, 25 aa, Rattus norvegicus
DVQLEESGGGLVRPGRSLKLSCADS

SEQ ID NO: 127 - protein, 8 aa, Rattus norvegicus
GVNFSNRG

SEQ ID NO: 128 - protein, 17 aa, Rattus norvegicus
MAWVRQAPTKGLEWVAT

SEQ ID NO: 129 - protein, 8 aa, Rattus norvegicus
ISYDGRII

SEQ ID NO: 130 - protein, 38 aa, Rattus norvegicus
YYRDSVKGRFSISRENAKSTLYLQMDSLRSEDTATYYC

SEQ ID NO: 131 - protein, 13 aa, Rattus norvegicus
ARHPIAADWYFDF

SEQ ID NO: 132 - protein, 11 aa, Rattus norvegicus
WGPGTMVTVSS

SEQ ID NO: 133 - protein, 25 aa, Rattus norvegicus
EVQLVESGGGSVQPGRSLKLSCAAS

SEQ ID NO: 134 - protein, 8 aa, Rattus norvegicus
GFTFSDYN

SEQ ID NO: 135 - protein, 17 aa, Rattus norvegicus
MAWVRQAPKKGPEWVAT

SEQ ID NO: 136 - protein, 8 aa, Rattus norvegicus
ITYDVHNA

SEQ ID NO: 137 - protein, 38 aa, Rattus norvegicus
YYRDSVKGRFTISRDDAKSTLYLQMDSLRSEDTATYFC

SEQ ID NO: 138 - protein, 6 aa, Rattus norvegicus
ARPGAY

SEQ ID NO: 139 - protein, 25 aa, Rattus norvegicus
QVRLLQSGAALVKPGASVKMSCKAS

SEQ ID NO: 140 - protein, 8 aa, Rattus norvegicus
GYTFTDYW

SEQ ID NO: 141 - protein, 17 aa, Rattus norvegicus
MSWVKQSHGKSLEWIGE

SEQ ID NO: 142 - protein, 8 aa, Rattus norvegicus
IYPNSGAT

SEQ ID NO: 143 - protein, 38 aa, Rattus norvegicus
NFNEKFKDKATLTVDRSTSTAYMELSRLTSEDSAIYYC

SEQ ID NO: 144 - protein, 14 aa, Rattus norvegicus
ARGFPNNYLSWFAY

SEQ ID NO: 145 - protein, 25 aa, Rattus norvegicus
QIQLVQSGPELKKPGESVKISCKAS

SEQ ID NO: 146 - protein, 8 aa, Rattus norvegicus
GYTFTNYG

SEQ ID NO: 147 - protein, 17 aa, Rattus norvegicus
MYWVKQAPGQGLQYMGW

SEQ ID NO: 148 - protein, 8 aa, Rattus norvegicus
INTETGKP

SEQ ID NO: 149 - protein, 38 aa, Rattus norvegicus
TYADDFKGRFVFFLETSASTAYLQINNLKNEDMATYFC

SEQ ID NO: 150 - protein, 14 aa, Rattus norvegicus
AREVKHGLFHWFAY

SEQ ID NO: 151 - protein, 25 aa, Rattus norvegicus
EVQLVESGGGLVQPGRSLTLSCSAS

SEQ ID NO: 152 - protein, 8 aa, Rattus norvegicus
GFTFRDYN

SEQ ID NO: 153 - protein, 17 aa, Rattus norvegicus
MAWVRQAPRKGLEWVAT

SEQ ID NO: 154 - protein, 8 aa, Rattus norvegicus
ISFDDYNT

SEQ ID NO: 155 - protein, 38 aa, Rattus norvegicus
YYRDSVKGRFTISRDDAKSTLYLQMDSLRSEDTATYYC

SEQ ID NO: 156 - protein, 6 aa, Rattus norvegicus
ARPGTY

SEQ ID NO: 157 - protein, 25 aa, Rattus norvegicus
QVQLQQSGAELVKPGSSVRISCKAS

SEQ ID NO: 158 - protein, 8 aa, Rattus norvegicus
GYTITSYD

SEQ ID NO: 159 - protein, 17 aa, Rattus norvegicus
MHWIKQQPGNGLEGIGW

SEQ ID NO: 160 - protein, 8 aa, Rattus norvegicus
IHPGNGKI

SEQ ID NO: 161 - protein, 38 aa, Rattus norvegicus
KYNQKFNGKATLTVDKSSSTAYMQLSSLTSEDSAVYFC

SEQ ID NO: 162 - protein, 13 aa, Rattus norvegicus
ARGTTRVFPWFAY

SEQ ID NO: 163 - protein, 8 aa, Rattus norvegicus
GFSFSNYG

SEQ ID NO: 164 - protein, 17 aa, Rattus norvegicus
MHWIRQAPTKGLEWVAS

SEQ ID NO: 165 - protein, 8 aa, Rattus norvegicus
ISPTGGNT

SEQ ID NO: 166 - protein, 38 aa, Rattus norvegicus
YYRDSVKGRFTISRDNTKSTLYLQMDSLRSEDTATYYC

SEQ ID NO: 167 - protein, 13 aa, Rattus norvegicus
ATDDLYYSGPFAY

SEQ ID NO: 168 - protein, 117 aa, Rattus norvegicus
EVQLQESGPGLVKPAQSLSLTCSVTGYSITNMYRWNWIRKFPGNKLEWMGYINTAGSTDYSPSLRGRVSITGDTSKNQFFLHLTSVTTEDTATYYCAGFITNPFDFWGQGVMVTVSS

SEQ ID NO: 169 - protein, 113 aa, Rattus norvegicus
EVQVVESGGGLVQPGRSLKLSCVPSGFTFNNYWMTWIRQAPGKAPEWVASISNTGGSTFYPDSVRGRFSISRDNTKGTLYLHMTSLRSEDTATYYCIRNMDAWGQGTSVTVSS

SEQ ID NO: 170 - protein, 122 aa, Rattus norvegicus
GKLVESGGGLLKPGGSLKLSCVASGFTFDKYWMHWVRQAPGKGLEWIAEIEYDGTETNYAPSIKDRFTISRDNAKNTLYLQMSNVRSEDAATYFCTTEEMYTTDYYYGFAYWGQGTLVTVSS

SEQ ID NO: 171 - protein, 123 aa, Rattus norvegicus
DVKLVESGGGLLKPGGSLKLSCVASGFSFSKYWMHWVRQAPGQGLEWIAEIEYDGTETNYAPSIKDRFTISRDNAKNTLYLQMSNVRFEDAATYFCTTEEMHTTDYYYGFAYWGQGTLVTVSS

SEQ ID NO: 172 - protein, 117 aa, Rattus norvegicus
EVQLVESGGGLVQPGRSLKLSCAASGFIFSEHNMAWVRQAPKKGLEWVATISDDGRNTYYRDSMRGRFTISRENARSTLYLQLDSLRSEDTATYYCASHRYNLFDSWGQGVMVTVSS

SEQ ID NO: 173 - protein, 114 aa, Rattus norvegicus
QVQLQQSGTELVKPASSVRISCKASGYTLTTNYMHWIRQQPGNGLEWIGWIYPGNGNTKFNHKFDGRTTLTADKSSSIVYMQLSSLTSEDSAVYFCARSDFDYWGQGVMVTVSS

SEQ ID NO: 174 - protein, 120 aa, Rattus norvegicus
DVQLEESGGGLVRPGRSLKLSCADSGVNFSNRGMAWVRQAPTKGLEWVATISYDGRIIYYRDSVKGRFSISRENAKSTLYLQMDSLRSEDTATYYCARHPIAADWYFDFWGPGTMVTVSS

SEQ ID NO: 175 - protein, 113 aa, Rattus norvegicus
EVQLVESGGGSVQPGRSLKLSCAASGFTFSDYNMAWVRQAPKKGPEWVATITYDVHNAYYRDSVKGRFTISRDDAKSTLYLQMDSLRSEDTATYFCARPGAYWGQGTLVTVSS

SEQ ID NO: 176 - protein, 121 aa, Rattus norvegicus
QVRLLQSGAALVKPGASVKMSCKASGYTFTDYWMSWVKQSHGKSLEWIGEIYPNSGATNFNEKFKDKATLTVDRSTSTAYMELSRLTSEDSAIYYCARGFPNNYLSWFAYWGQGTLVTVSS

SEQ ID NO: 177 - protein, 121 aa, Rattus norvegicus
QIQLVQSGPELKKPGESVKISCKASGYTFTNYGMYWVKQAPGQGLQYMGWINTETGKPTYADDFKGRFVFFLETSASTAYLQINNLKNEDMATYFCAREVKHGLFHWFAYWGQGTLVTVSS

SEQ ID NO: 178 - protein, 113 aa, Rattus norvegicus
EVQLVESGGGLVQPGRSLTLSCSASGFTFRDYNMAWVRQAPRKGLEWVATISFDDYNTYYRDSVKGRFTISRDDAKSTLYLQMDSLRSEDTATYYCARPGTYWGQGTLVTVSS

SEQ ID NO: 179 - protein, 120 aa, Rattus norvegicus
QVQLQQSGAELVKPGSSVRISCKASGYTITSYDMHWIKQQPGNGLEGIGWIHPGNGKIKYNQKFNGKATLTVDKSSSTAYMQLSSLTSEDSAVYFCARGTTRVFPWFAYWGQGTLVTVSS

SEQ ID NO: 180 - protein, 120 aa, Rattus norvegicus
EVQLVESGGGLVQPGRSLKLSCAASGFSFSNYGMHWIRQAPTKGLEWVASISPTGGNTYYRDSVKGRFTISRDNTKSTLYLQMDSLRSEDTATYYCATDDLYYSGPFAYWGQGTLVTVSS

SEQ ID NO: 181 - protein, 25 aa, Homo sapiens [sequence omitted]

SEQ ID NO: 182 - protein, 17 aa, Homo sapiens
MHWVRQAPGQRLEWMGW

SEQ ID NO: 183 - protein, 38 aa, Homo sapiens
KFNHKFDGRVTITRDTSASTAYMELSSLRSEDTAVYYC

SEQ ID NO: 184 - protein, 17 aa, Homo sapiens
MHWVRQAPGQGLEWMGW

SEQ ID NO: 185 - protein, 38 aa, Homo sapiens
KFNHKFDGRVTMTRDTSTSTVYMELSSLRSEDTAVYYC

SEQ ID NO: 186 - protein, 11 aa, Homo sapiens
WGQGTMVTVSS

SEQ ID NO: 187 - protein, 38 aa, Homo sapiens
KFNHKFDGRVTMTRDTSISTAYMELSRLRSDDTAVYYC

SEQ ID NO: 188 - protein, 25 aa, Homo sapiens [sequence omitted]

SEQ ID NO: 189 - protein, 38 aa, Homo sapiens
KFNHKFDGRVTITADKSTSTAYMELSSLRSEDTAVYYC

SEQ ID NO: 190 - protein, 25 aa, Homo sapiens
QVQLVQSGSELKKPGASVKVSCKAS

SEQ ID NO: 191 - protein, 38 aa, Homo sapiens
KFNHKFDGRFVFSLDTSVSTAYLQISSLKAEDTAVYYC

SEQ ID NO: 192 - protein, 114 aa, Artificial sequence
  Humanised heavy chain variable region
QVQLVQSGAEVKKPGASVKVSCKASGYTLTTNYMHWVRQAPGQRLEWMGWIYPGNGNTKFNHKFDGRVTITRDTSASTAYMELSSLRSEDTAVYYCARSDFDYWGQGTLVTVSS

SEQ ID NO: 193 - protein, 114 aa, Artificial sequence
  Humanised heavy chain variable region
QVQLVQSGAEVKKPGASVKVSCKASGYTLTTNYMHWVRQAPGQGLEWMGWIYPGNGNTKFNHKFDGRVTMTRDTSTSTVYMELSSLRSEDTAVYYCAISDFDYWGQGTMVTVSS

SEQ ID NO: 194 - protein, 114 aa, Artificial sequence
  Humanised heavy chain variable region
QVQLVQSGAEVKKPGASVKVSCKASGYTLTTNYMHWVRQAPGQGLEWMGWIYPGNGNTKFNHKFDGRVTMTRDTSISTAYMELSRLRSDDTAVYYCARSDFDYWGQGTLVTVSS

SEQ ID NO: 195 - protein, 114 aa, Artificial sequence
  Humanised heavy chain variable region
QVQLVQSGAEVKKPGSSVKVSCKASGYTLTTNYMHWVRQAPGQGLEWMGWIYPGNGNTKFNHKFDGRVTITADKSTSTAYMELSSLRSEDTAVYYCATSDFDYWGQGTLVTVSS

SEQ ID NO: 196 - protein, 114 aa, Artificial sequence
  Humanised heavy chain variable region
QVQLVQSGSELKKPGASVKVSCKASGYTLTTNYMHWVRQAPGQGLEWMGWIYPGNGNTKFNHKFDGRFVFSLDTSVSTAYLQISSLKAEDTAVYYCARSDFDYWGQGTLVTVSS

SEQ ID NO: 197 - protein, 26 aa, Homo sapiens
DIQMTQSPSSLSASVGDRVTITCQAS

SEQ ID NO: 198 - protein, 17 aa, Homo sapiens
LIWFQQKPGKAPKSLIY

SEQ ID NO: 199 - protein, 36 aa, Homo sapiens
SLANGVPSRFSGSGSGTDFTLTISSLQPEDFATYYC

SEQ ID NO: 200 - protein, 10 aa, Homo sapiens
FGPGTKVDIK

SEQ ID NO: 201 - protein, 26 aa, Homo sapiens
DIQMTQSPSAMSASVGDRVTITCQAS

SEQ ID NO: 202 - protein, 17 aa, Homo sapiens
LIWFQQKPGKVPKRLIY

SEQ ID NO: 203 - protein, 36 aa, Homo sapiens
SLANGVPSRFSGSGSGTEFTLTISSLQPEDFATYYC

SEQ ID NO: 204 - protein, 17 aa, Homo sapiens
LIWYQQKPGKAPKRLIY

SEQ ID NO: 205 - protein, 10 aa, Homo sapiens
FGQGTKLEIK

SEQ ID NO: 206 - protein, 17 aa, Homo sapiens
LIWYQQKPGKAPKLLIY

SEQ ID NO: 207 - protein, 36 aa, Homo sapiens
SLANGVPSRFSGSGSGTDFTFTISSLQPEDIATYYC

SEQ ID NO: 208 - protein, 26 aa, Homo sapiens
DIQMTQSPSSVSASVGDRVTITCQAS

SEQ ID NO: 209 - protein, 10 aa, Homo sapiens
FGQGTKVEIK

SEQ ID NO: 210 - protein, 107 aa, Artificial sequence
  Humanised light chain variable region
DIQMTQSPSSLSASVGDRVTITCQASQDIGNNLIWFQQKPGKAPKSLIYFATSLANGVPSRFSGSGSGTDFTLTISSLQPEDFATYYCLQYREYPLTFGPGTKVDIK

SEQ ID NO: 211 - protein, 107 aa, Artificial sequence
  Humanised light chain variable region
DIQMTQSPSAMSASVGDRVTITCQASQDIGNNLIWFQQKPGKVPKRLIYFATSLANGVPSRFSGSGSGTEFTLTISSLQPEDFATYYCLQYREYPLTFGPGTKVDIK

SEQ ID NO: 212 - protein, 107 aa, Artificial sequence
  Humanised light chain variable region
DIQMTQSPSSLSASVGDRVTITCQASQDIGNNLIWYQQKPGKAPKRLIYFATSLANGVPSRFSGSGSGTEFTLTISSLQPEDFATYYCLQYREYPLTFGQGTKLEIK

SEQ ID NO: 213 - protein, 107 aa, Artificial sequence
  Humanised light chain variable region
DIQMTQSPSSLSASVGDRVTITCQASQDIGNNLIWYQQKPGKAPKLLIYFATSLANGVPSRFSGSGSGTDFTFTISSLQPEDIATYYCLQYREYPLTFGQGTKLEIK

SEQ ID NO: 214 - protein, 107 aa, Artificial sequence
  Humanised light chain variable region
DIQMTQSPSSVSASVGDRVTITCQASQDIGNNLIWYQQKPGKAPKLLIYFATSLANGVPSRFSGSGSGTDFTLTISSLQPEDFATYYCLQYREYPLTFGQGTKVEIK

SEQ ID NO: 215 - protein, 25 aa, Homo sapiens
QVQLVESGGGVVQPGRSLRLSCAAS

SEQ ID NO: 216 - protein, 17 aa, Homo sapiens
MAWVRQAPGKGLEWVAT

SEQ ID NO: 217 - protein, 38 aa, Homo sapiens
YYRDSMRGRFTISRDNSKNTLYLQMNSLRAEDTAVYYC

SEQ ID NO: 218 - protein, 25 aa, Homo sapiens [sequence omitted]

SEQ ID NO: 219 - protein, 17 aa, Homo sapiens
MAWVRQAPGKGLEWVST

SEQ ID NO: 220 - protein, 38 aa, Homo sapiens
YYRDSMRGRFTISRDNAKNSLYLQMNSLRAEDTAVYYC

SEQ ID NO: 221 - protein, 17 aa, Homo sapiens
MAWVRQAPGKGLVWVST

SEQ ID NO: 222 - protein, 38 aa, Homo sapiens
YYRDSMRGRFTISRDNAKNTLYLQMNSLRAEDTAVYYC

SEQ ID NO: 223 - protein, 25 aa, Homo sapiens [sequence omitted]

SEQ ID NO: 224 - protein, 38 aa, Homo sapiens
YYRDSMRGRFTISRDNAKNSLYLQMNSLRAEDTALYYC

SEQ ID NO: 225 - protein, 117 aa, Artificial sequence
  Humanised heavy chain variable region
QVQLVESGGGVVQPGRSLRLSCAASGFIFSEHNMAWVRQAPGKGLEWVATISDDGRNTYYRDSMRGRFTISRDNSKNTLYLQMNSLRAEDTAVYYCTSHRYNLFDSWGQGTMVTVSS

SEQ ID NO: 226 - protein, 117 aa, Artificial sequence
  Humanised heavy chain variable region
EVQLVESGGGLVQPGGSLRLSCAASGFIFSEHNMAWVRQAPGKGLEWVSTISDDGRNTYYRDSMRGRFTISRDNSKNTLYLQMNSLRAEDTAVYYCAKHRYNLFDSWGQGTLVTVSS

SEQ ID NO: 227 - protein, 117 aa, Artificial sequence
  Humanised heavy chain variable region
EVQLVESGGGLVQPGGSLRLSCAASGFIFSEHNMAWVRQAPGKGLEWVATISDDGRNTYYRDSMRGRFTISRDNAKNSLYLQMNSLRAEDTAVYYCARHRYNLFDSWGQGTMVTVSS

SEQ ID NO: 228 - protein, 117 aa, Artificial sequence
  Humanised heavy chain variable region
EVQLVESGGGLVQPGGSLRLSCAASGFIFSEHNMAWVRQAPGKGLVWVSTISDDGRNTYYRDSMRGRFTISRDNAKNTLYLQMNSLRAEDTAVYYCARHRYNLFDSWGQGTLVTVSS

SEQ ID NO: 229 - protein, 117 aa, Artificial sequence
  Humanised heavy chain variable region
EVQLVESGGGLVQPGRSLRLSCAASGFIFSEHNMAWVRQAPGKGLEWVSTISDDGRNTYYRDSMRGRFTISRDNAKNSLYLQMNSLRAEDTALYYCAKHRYNLFDSWGQGTLVTVSS

SEQ ID NO: 230 - protein, 26 aa, Homo sapiens [sequence omitted]

SEQ ID NO: 231 - protein, 17 aa, Homo sapiens
LNWYQQKPGKAPKRLIY

SEQ ID NO: 232 - protein, 36 aa, Homo sapiens
KLQTGVPSRFSGSGSGTEFTLTISSLQPEDFATYYC

SEQ ID NO: 233 - protein, 17 aa, Homo sapiens
LNWFQQKPGKAPKSLIY

SEQ ID NO: 234 - protein, 36 aa, Homo sapiens
KLQTGVPSKFSGSGSGTDFTLTISSLQPEDFATYYC

SEQ ID NO: 235 - protein, 10 aa, Homo sapiens
FGQGTRLEIK

SEQ ID NO: 236 - protein, 17 aa, Homo sapiens
LNWYQQKPGKAPKLLIY

SEQ ID NO: 237 - protein, 36 aa, Homo sapiens
KLQTGVPSRFSGSGSGTDFTLTISSLQPEDFATYYC

SEQ ID NO: 238 - protein, 26 aa, Homo sapiens
DIQLTQSPSFLSASVGDRVTITCKAS

SEQ ID NO: 239 - protein, 26 aa, Homo sapiens
DIQMTQSPSTLSASVGDRVTITCKAS

SEQ ID NO: 240 - protein, 36 aa, Homo sapiens
KLQTGVPSRFSGSGSGTEFTLTISSLQPDDFATYYC

SEQ ID NO: 241 - protein, 107 aa, Artificial sequence
  Humanised light chain variable region
DIQMTQSPSSLSASVGDRVTITCKASQNIDRYLNWYQQKPGKAPKRLIYNTNKLQTGVPSRFSGSGSGTEFTLTISSLQPEDFATYYCLQYNSLPLTFGQGTKLEIK

SEQ ID NO: 242 - protein, 107 aa, Artificial sequence
  Humanised light chain variable region
DIQMTQSPSSLSASVGDRVTITCKASQNIDRYLNWFQQKPGKAPKSLIYNTNKLQTGVPSKFSGSGSGTDFTLTISSLQPEDFATYYCLQYNSLPLTFGQGTRLEIK

SEQ ID NO: 243 - protein, 107 aa, Artificial sequence
  Humanised light chain variable region
DIQMTQSPSSLSASVGDRVTITCKASQNIDRYLNWYQQKPGKAPKLLIYNTNKLQTGVPSRFSGSGSGTDFTLTISSLQPEDFATYYCLQYNSLPLTFGQGTKLEIK

SEQ ID NO: 244 - protein, 107 aa, Artificial sequence
  Humanised light chain variable region
DIQLTQSPSFLSASVGDRVTITCKASQNIDRYLNWYQQKPGKAPKLLIYNTNKLQTGVPSRFSGSGSGTEFTLTISSLQPEDFATYYCLQYNSLPLTFGQGTKLEIK

SEQ ID NO: 245 - protein, 107 aa, Artificial sequence
  Humanised light chain variable region
DIQMTQSPSTLSASVGDRVTITCKASQNIDRYLNWYQQKPGKAPKLLIYNTNKLQTGVPSRFSGSGSGTEFTLTISSLQPDDFATYYCLQYNSLPLTFGQGTKLEIK

SEQ ID NO: 246 - protein, 7 aa, Artificial sequence
  Humanised heavy chain CDR3
AISDFDY

SEQ ID NO: 247 - protein, 7 aa, Artificial sequence
  Humanised heavy chain CDR3
ATSDFDY

SEQ ID NO: 248 - protein, 7 aa, Artificial sequence
  Humanised heavy chain CDR3
  misc_feature (2)..(2): Xaa can be Arg, Ile or Thr
AXSDFDY

SEQ ID NO: 249 - protein, 10 aa, Artificial sequence
  Humanised heavy chain CDR3
TSHRYNLFDS

SEQ ID NO: 250 - protein, 10 aa, Artificial sequence
  Humanised heavy chain CDR3
AKHRYNLFDS

SEQ ID NO: 251 - protein, 10 aa, Artificial sequence
  Humanised heavy chain CDR3
ARHRYNLFDS

SEQ ID NO: 252 - protein, 10 aa, Artificial sequence
  Humanised heavy chain CDR3
  misc_feature (1)..(1): Xaa can be Ala or Thr
  misc_feature (2)..(2): Xaa can be Ser, Lys or Arg
XXHRYNLFDS

SEQ ID NO: 253 - protein, 5 aa, Homo sapiens
NISSE

SEQ ID NO: 254 - protein, 5 aa, Artificial sequence
  Substituted sequence for epitope mapping
FQDDL

SEQ ID NO: 255 - protein, 16 aa, Rattus norvegicus
RSSQSLEHSNGDTFLH

SEQ ID NO: 256 - protein, 7 aa, Rattus norvegicus
RVSNRFS

SEQ ID NO: 257 - protein, 6 aa, Rattus norvegicus
NMYRWN

SEQ ID NO: 258 - protein, 16 aa, Rattus norvegicus
YINTAGSTDYSPSLRG

SEQ ID NO: 259 - protein, 8 aa, Rattus norvegicus
FITNPFDF

SEQ ID NO: 260 - protein, 11 aa, Rattus norvegicus
RASQSISNSLN

SEQ ID NO: 261 - protein, 7 aa, Rattus norvegicus
STSTLES

SEQ ID NO: 262 - protein, 5 aa, Rattus norvegicus
NYWMT

SEQ ID NO: 263 - protein, 17 aa, Rattus norvegicus
SISNTGGSTFYPDSVRG

SEQ ID NO: 264 - protein, 4 aa, Rattus norvegicus
NMDA

SEQ ID NO: 265 - protein, 15 aa, Rattus norvegicus
RASQSVSISRYNFMH

SEQ ID NO: 266 - protein, 7 aa, Rattus norvegicus
RASNLAS

SEQ ID NO: 267 - protein, 5 aa, Rattus norvegicus
KYWMH

SEQ ID NO: 268 - protein, 17 aa, Rattus norvegicus
EIEYDGTETNYAPSIKD

SEQ ID NO: 269 - protein, 14 aa, Rattus norvegicus
EEMYTTDYYYGFAY

SEQ ID NO: 270 - protein, 15 aa, Rattus norvegicus
RASQSVSISRYDFMH

SEQ ID NO: 271 - protein, 14 aa, Rattus norvegicus
EEMHTTDYYYGFAY

SEQ ID NO: 272 - protein, 11 aa, Rattus norvegicus
KASQNIDRYLN

SEQ ID NO: 273 - protein, 7 aa, Rattus norvegicus
NTNKLQT

SEQ ID NO: 274 - protein, 5 aa, Rattus norvegicus
EHNMA

SEQ ID NO: 275 - protein, 17 aa, Rattus norvegicus
TISDDGRNTYYRDSMRG

SEQ ID NO: 276 - protein, 8 aa, Rattus norvegicus
HRYNLFDS

SEQ ID NO: 277 - protein, 11 aa, Rattus norvegicus
QASQDIGNNLI

SEQ ID NO: 278 - protein, 7 aa, Rattus norvegicus
FATSLAN

SEQ ID NO: 279 - protein, 5 aa, Rattus norvegicus
TNYMH

SEQ ID NO: 280 - protein, 17 aa, Rattus norvegicus
WIYPGNGNTKFNHKFDG

SEQ ID NO: 281 - protein, 5 aa, Rattus norvegicus
SDFDY

SEQ ID NO: 282 - protein, 11 aa, Rattus norvegicus
LTSEDIYSDLA

SEQ ID NO: 283 - protein, 7 aa, Rattus norvegicus
DANSLQN

SEQ ID NO: 284 - protein, 5 aa, Rattus norvegicus
NRGMA

SEQ ID NO: 285 - protein, 17 aa, Rattus norvegicus
TISYDGRIIYYRDSVKG

SEQ ID NO: 286 - protein, 11 aa, Rattus norvegicus
HPIAADWYFDF

SEQ ID NO: 287 - protein, 11 aa, Rattus norvegicus
QSSQGIGKYLS

SEQ ID NO: 288 - protein, 7 aa, Rattus norvegicus
YATKLAD

SEQ ID NO: 289 - protein, 5 aa, Rattus norvegicus
DYNMA

SEQ ID NO: 290 - protein, 17 aa, Rattus norvegicus
TITYDVHNAYYRDSVKG

SEQ ID NO: 291 - protein, 4 aa, Rattus norvegicus
PGAY

SEQ ID NO: 292 - protein, 15 aa, Rattus norvegicus
KTSQNVDNHGISYMH

SEQ ID NO: 293 - protein, 7 aa, Rattus norvegicus
EGSNLAV

SEQ ID NO: 294 - protein, 5 aa, Rattus norvegicus
DYWMS

SEQ ID NO: 295 - protein, 17 aa, Rattus norvegicus
EIYPNSGATNFNEKFKD

SEQ ID NO: 296 - protein, 12 aa, Rattus norvegicus
GFPNNYLSWFAY

SEQ ID NO: 297 - protein, 13 aa, Rattus norvegicus
ERSSGDIGDSYVS

SEQ ID NO: 298 - protein, 7 aa, Rattus norvegicus
ADDQRPS

SEQ ID NO: 299 - protein, 5 aa, Rattus norvegicus
NYGMY

SEQ ID NO: 300 - protein, 17 aa, Rattus norvegicus
WINTETGKPTYADDFKG

SEQ ID NO: 301 - protein, 12 aa, Rattus norvegicus
EVKHGLFHWFAY

SEQ ID NO: 302 - protein, 7 aa, Rattus norvegicus
YATNLAD

SEQ ID NO: 303 - protein, 17 aa, Rattus norvegicus
TISFDDYNTYYRDSVKG

SEQ ID NO: 304 - protein, 4 aa, Rattus norvegicus
PGTY

SEQ ID NO: 305 - protein, 12 aa, Rattus norvegicus
ERSSGDIGDNYV

SEQ ID NO: 306 - protein, 5 aa, Rattus norvegicus
SYDMH

SEQ ID NO: 307 - protein, 17 aa, Rattus norvegicus
WIHPGNGKIKYNQKFNG

SEQ ID NO: 308 - protein, 11 aa, Rattus norvegicus
GTTRVFPWFAY

SEQ ID NO: 309 - protein, 11 aa, Rattus norvegicus
KASQNITRFLN

SEQ ID NO: 310 - protein, 7 aa, Rattus norvegicus
NTNNLQT

SEQ ID NO: 311 - protein, 5 aa, Rattus norvegicus
NYGMH

SEQ ID NO: 312 - protein, 17 aa, Rattus norvegicus
SISPTGGNTYYRDSVKG

SEQ ID NO: 313 - protein, 11 aa, Rattus norvegicus
DDLYYSGPFAY